European Patent Application EP 4 230 749 A1, published August 23, 2023. Title: In vitro method for predicting a risk of post-chikungunya chronic inflammatory joint disease. Applicant: BIOMERIEUX UNIVERSIDADE DE SAO PAULO. The sequence listing filed with the application follows.

SEQUENCE LISTING (8 sequences)

SEQ ID NO: 1 - RNA, 2728 nt, Homo sapiens
aggaccgccgagcuuugcugaggcaucauggugggacuuaaagaaguaucuuggccgggcgcaguggcucacaccuauaaucccagaacuuugggaggaugaggcaggaggaucaauugagucacggaguucaagaccagccugggcaacagagugagacucugucucuacaacaaauuuuaaaaaaauuagucagguauggugacgugcacguauagucucagcuacuugggaggcugaggugggaggaucacuugagcucgggagguggagguugcagugagccaugauugcgccacucacucuaacauaggugacagagugagaucccgucuccaaaaacaaacacaaacaaacuaaaagaaguaucagcugcuacacaucuggaaugacaacauaugcagaauacaaauguaaauagaaaacauagaauauaaauuaugaguuuuaguugaguaacgcugacuuggaauuggaagaacauuugcaggcaucaguaaugggagaguagaaaaugugagaaagaaaccuuaagucaauuaagagaauacacucugcaaauuagggguggauccuuggguuaaucugcagccugcaguuguacccugcuagaagcagcuucgaugccacugaaguuaaucuugggucccaguaaauaucuucucuccucucuauuauccacugugcaagauauauguaaauacugccagauacauuuuuuaaaaggcccgggugcuaucguguauagguugacauuaauguacucccagaaugcccaggcaugguaugggguggccacccuaugguuccuguuuucuuagacggaagaccacuccugcagaacauuuauuaucagccuaggccagugugaacauacuggguacauuuuaggauucaguuuaucuguuuuguuuaggguuggugcuaauuuggaauaagcaaaccauucaugaucuguaucacauaauuugguuuagaaucugucaccuuaccuguugcggucacucccucugaauuuggggaccccaagaccaaguuuuacucuucugcucuuuccaccuccagugcuaaggccuagaggggcgcaccuuaaaucugaaucaauccacaaagcccgacggacgccaguggcaggguuuggugggauuuuaauaguaaccuacaaaaaaagucaggaagauagggaauagggacgaauuauucucuucuacucuucaaauuuucaguguugcucucauugcauauucucaccuugaaaucacugcuagagacuucccaaguccaaaggguaagaaacuaccuucagacuggcuugggaaauguuuagagcugccaggguuguauguaaaauuuccauggcaauaaaccacugauacauuuuuuguucuauuccaccuaggaaaaacaaagauccccaaaguccauuucgcuccgaggucaguggacacagcucugugacuguccugugcugugugggucuguagaagggccagucaugggccaucgagcuacucacagccaacugcacccaaguccaagccuggcucuguucccauacacagagacaggaugggggcugcugaucuggccugaagccuugcucugggcacugaaaacgggggcuauuuccuuaccugaagaucuggaagcagcauguugacaaaagcaccaacugcucugccaucacgucccacugggugucagugggaaggccuaaccaaggccugccuccaguggcuaucaggcagacgggccagcaguuccccuccaggagcaagggacccuucuuacccuuuugaucacauuucccucucuuaaaggggcacugcugugggaaggggucaugccuuggauccuacagucauggacugugggugaaacaggggcucuugacucuucacuuccuagccauaacucugcccauuggaccacccacccucccugcugcuggucuccuggcucacccaucaaauccaacugcuuuaucuagaaaauacuuuucuccauucucauuucccuuugcuuucccacucaccucuguuuuuguuucuguuuuauuuuguuccagacacccuuuucagggaaguagaucagggaggcccaagagauuaggccugggugggcugcuaucgcuuaagaacacgucugccucuggggcuccucccuaacagcuggccucuggagcugggagaugcagcugccuggcagucugcagaggcagauuguguuguuacgugcuggucaccgccuugagccuuaaaccacagucagcaaugaaccuggaggcagggcaucucuggggaugaucgaccgcaucugcucagguucuugcagggcagggcaggcagagauguguguuuggagccagaaagccuuccugccaaccugccaugccucaguuucccuaucugaaccaccuucauaaaaacaacuuacggcucucagagcagcacauuuguaaaaaccugaaaaauauaaagaaaaacgucacucacauuucucccaugaacauuuuccuauuuuauguaucuuuuauguaacugaaucacauugcauauacaauuauguguuccauuuuuaaacaauaagcuucccuuguuuuaaaaguaauaauccauguuuauuauguguuauugcauagaaauuucagacacaaaaaaagaaaggaaaaaugacuccuuauugcuccauugagaaauaauaaauaugaauauuauucugauaaaua

SEQ ID NO: 2 - RNA, 8559 nt, Homo sapiens
aauuuuuuuuuuuuuuuuuuuuuugagagaaagucucacucuguugcccaggcuagagugcagugguacagucuuggcucacugcaaccucugccucccagguucaagcgauucuugugucucagccucccaaguaguugagauuacaggcacgagccaccacaccuggcgaauuuuuguauuuuuaguagagaggggguuucaccauguuggccaggcuggucucaacuccugaccucaaguaauccacccaucucagccucccaaagugcugggauuacaggcgugagccacagcaccugcccugguuguccuacuuucaaugaugcuaagauuaaucaguguuucaggugauaacagacugauccuuccauuguaaagcuccaaucaacauuuugucuaaugauuuuagccauuaauaaucauacccuaagucaauuacaugcugcaaaugaugauuagauucuauuauuuuuucauuaucuauuuucuuugacauucauuagcuugaauucuauaaagaagaacuuuuccuucuaaguuaaggcuaugugguuacacauacaugccuaaaagaaagcagaauaaagauaaguauuuauuuugauugccaaauaucaggguaaggaguaacugaccuaguuaauucuaauggugaccaaagugugaugacuuuuaaacauuuuauugauuuucuuuuuuguaucuuuauaauuaaugcauuuugaaauaaauucaacacauuuaaaucaauugcauucaguauauguuuucucuuuugacucucaucuugccuccaguuuggcuaaagaaagacuuuuuagguuaauuccuuuguccuuugggcacaaucucauuagucuuugauagcuaccuugcuuucuaagugauaugguuaggcuuugugucccuacccaaaucucaucuugaauuguaauccccauaauccccaucauccccacguguaaagggagagacgagauagagguaacaaucaugguggcaguuucucucaugcuguucucaugauagugaguucucacaagaucugaugguuuuauaaagagcucuucccccuucacuuggcauuguccuucuugccaccacuuugugaagaaggugccuugcuuccccuuugccuucuaccaugauuuuaaguuuucugaggccuccccagccacacugaacugugagucaauuaaaccucuuuucuucauaaauuacccaguuucuggcaguuccuuauagcagugugaaaacagacuaauacaccagggcaacaaaccgucccaggcucaucuuaaauugccuaaccuuaaaacuggagucaggugucccuccaaaguuuccuagucauuguuaguguggaaugguauuuagggauuauagucuauaugcuaaguaugcucauuuucaagggguuguagaauaguuuauauuauuauccucaacuccuaacucccuucucauuuauuauuguaugauuucuagggccucccagcaggcagaacacaauucuccaucccaguuccacguuuggccacgugaugugcuuugaccaaugggcacauaucauguuaaguagaagcuuuuagagcuguuaaggacagagcuaagcuuuguccuuugcuuuucccuaggccacaaggacagucuguuccaaacagggucaauugcuucagcuugaguccuggaaaaagaagauuguagagaaaagacucagcagcugaucuggagccaccaaaauggaauacaagccaaauauauaaugcauaugguggcaaacuacugagguuuuuaagguuaucuguuacuucuucaaagcugauugauacaggcugugaugucuucugggccuuuuuaguagacagauaggaaaagcagcuuugaaaagaggaaagcauugugaguucaaacucaauucaaauagaacauuuccaaaucagauagaacauuauaggaccuguacuuaauuuuuaaaaacuuuauacauauaucucuuuuuucuacacuaaaaaucuuaauuucuauuuacauuaguauaauuacugauuuguauuuccuauaauauaacauagugucaaaauaacaaaaucauuauuuuaaaguacuaaaguuuaaaacauauuuguagcuauuuuuguccuuaagauauauucuacuguuugguggaauauuauguuuuuagguucagauugaaauaauuauuuccuuuaugugguuauaucacuaauuugauauacaguagguucauuuccuuauuucuuuuuuuuucuuuuagagacagcaucuuucucugucacccacgcuagagugcaguagcacaaucacagcucaccacagccucgaucucccaggaccaagcaaaccucccaccucagccucgugaguagcugagacuacaggcaugccaccaugcccagcuaauuuuuauuuauuuuucuuuuuuguagaggcguggccuuccuauauggccuaggcuggucuugaacuccuggucuuaagcaaucuuccugccugggccucccaaaguauggggauuacaaguguaaaccaccaugcccagcucaguaaguucauuuauuuccauuuguuuuccauuuuuagggaaggcuauuuuagugaauuuuaucuuuugaaauaaaacauuuaaaauuucaaaaugaaaucuauguaauaagcuauacauaguaagagaagucuguuccauuccuguucuaccuauuguuaauaguuucauuaguuaacaguuuaaccugccaguguuucugucauacacaaaauguagcauguugcacuagauuguucugcaucuuacuuuuuucacuuacuauauuuuggagaugacaguacagagagaucaccaucauuccuuuauaucgcuacagugccuaccauuguguuauuuauuuagccaauccccuauaaaugggcauuuguuuucaaucauuuuuauaauaguugugaaauaaauaauacaaugcauaaaaaagaaauaacaccaugcauaaagcauguccuguuuuugcaacuacagcuuuaacacagguucccaguaacgggguugaugggucaaagggcaaauauagaauuuuucuacauauugcugaauaugaugggucaaaggcuagauguagaauuuuucuacauauugcugcuccauagcaguuguaucaucucacagcuccaucagcaguauguagaaugccuauuuccauacaacuucaauaacagaguauguggaugaguuuaugugauuuugcuaagggaagaagugcuaucuuugggacaaucuaauuugcauuuuaaguuauacugagaaaagcuucauauuugaagaaccauuuaaauuuuucuucugggaacucuggguuuuuugugugccauuuauaaaauuuugauauuuguauuuuaauuuuuagggguuccuuuuauaucagugauaauacucugucagagauguaacuuacaaauauccuuucccaauuagucauuuaucuuuggauuuguuuaggguguuuuauuuuuuccaugcagacacucauuugauuuauaguccaguuuacagaagaacagauccauacuuuguuuuuuuuuuuuuuuuuuuuuuggcggggggagguaugguuuuauuuauuuauuuaccuauuuacauuuagaucucugauccauuugaaauuaauucucauggagaauaucagguucugauccauuuuucccucaaaugguucccaguuguaacaauauugauuaagcauucuccaugguuucaaaugcuaccauuuuacacacacauacacacauacacgugauuucuaaaugaaguuggcauaauuuccggacuuuauauacucuuccauuggcuugucugucuauucauguaccaaucucacauuauuuuacuuauagaggcuuuauagaacacuauaauauagggcuauaaccacuucauuucugccccguuaguguauuauuaauucuccauugucucauucauuugauauuuauucuauguauuauauguuuuaugauuaauauguugauacagaaauacauauuacaauuuauuaaaacacacgucaggacauauccucuuuuaagaaaugaaguaggauauguaauauaaaaaaguuugaagaucacugauucaguguuuuuugaacaugccagcaucuuuagauagcuguccuggguggcaguagcacaauggagcugagauucuuacauguaucugauuuuggcauuugccuaaugcugaaugagauucuuggcagagacaaugacucaccuggauccagggguaauuuuuuaagugcuaaugagcaagugucaagaucccacaaaaucauuaaaaguaacggcuaaaacugcaguuacuuuugcaccaaccuauaaaaauacuggacaagaacaccuaggaaaaucaucuuugauuuggaaaugaagaucacuuuaucaggcucuacaaugguuuaaauguguuccucagaauucauguauaggaaauugaguucccaguauaaugguguugagaggugguaggaccuuuaagagguguuugggucaugaagacucugccacccucacgaagauauuagucccauucucauaggacuggguuaauucucacagaagcaaaugaguucuuguucucaugggacuagauuaguaacugcaagagcagguuguuaaaaaaugaggccaucacuuguguuuugucucuuuugcacauacuugcuugcugcuccugcagguguuuccacaugugaugccauucacuaugcuuuaauguagcaugagggccuugccagagguagcugcccaauguugaacuucccaggcuccagaacugggagccaaguaaaccucuuuuguuuauaaauuacccagucucagguguucuguuacagcaacagaaauagacuaaaacagucucuauugucucaucucucuuaauaaacuuuugcucauuaugggauauagauugcuauuauaucaauugaguaacaaagagauuaggccaugaggggaaagucuggagauucccugcuccagagaguagaacuuuuacaacuaacaugcuaauacgguuugguugugucgccacccaaaucucaucuugaauuguaguucccauaauccccacauguugugggagagacacgguggcagguaauugaaucauggaagugguuaccuccaugcuuucuuuucucaugauagugaaugagcucuuaugagaucugaugauuuuauaaagggcuuuccccgcuuuugcucggcacuucugcuuccggccaucaaguaaagaagaauguguuugcuuccccuucugccaugauuguaaguuuccugaggccuccccagccaugcgaaacugagagucaauuaaaccucuuuccuuuguaaauuacccagucuugggcaguccuuuacagcagcgugagaacacacuaauacgugcuuuguucuagucuagauuaagcaacuuuugagggguguauuguuugacucaucugaguuuuuaaucaaugcuuacuaauucaagaggaacuuaugugcuuuuaggauauaaggaggcaucaggaaaucuggaaaauuucuuaaaauccuauaaggcagaccagucuuuauauuuccuuauaucuuagggaggccacuguuaaaaagaggaggagggaguuuuaggagcaguaauauuaugcauucauuugagacuauuaauuuuacauaugucuugagguuuuuauugcuaaaaaguuauauaauuuuaugaagcuacaaaacaaauaaacauuaaauuccagcuuauguaauucuacuuaaucaaguauuaaaugugccaggcaguacucuagguaccaacgaccuaaagauguguugucucugccuccagcaagcucacaauacagagagauauacauggaaaaauuguaacaguacagcucaguaagugccauaagagaauaaagaauauaccaaaagcaccagaguauaauauacaguagacaucagcuuugaggaauugaugaguuggaaagaauuaagagaaggcgcaaggaauuuuggaguuagaccuucagggagaaauugcauuuggccauaugaggaacaauagcaacaacaacagagaugaauggagguugggaagaaguacuguaucuagauaaaauggcauagauguucacucguuuacacacacacacacacacacacacacaaacacacggcacaaaagaaccugacuuguucuggauccaaaagcacuauauggacaguacaauaaucucaugucuccaauaugcuuagguacaauuuuaauguuuuaugacauagauggcugcauguuucaguuauuggacaaaugcauacuugaguuauuguuuauuccauugugucaguucugcuucugaucaaaauccauuccuauuugaaaaugcaucuagugaauuuuuuuuuuugagacagaaucuugcuguguugcccaggcuggagugcaguggcacaaucucagcucauugcaaccuccgccucccacguucaagugauucucaugccucagccuccugaguagcugggacuacaggugcaugccaccaugcccagcuacuuuuuguacuuuuaguagauacaggguuucaccacguuggcuaggcugguuucaaacuccugaccucaggugauccacccgucuuggccucccaaagugcugggauuacaggcgugagucacagcgcccagcccucuagugcauuuuuuaaaaaacauaaacaccauucucucuuuucaaauuuagcacuugcccagaaguuugacauguucccuuuuuauuuguggucauuauuuccucuuuggucuccuuuaaaaauagcaccccuuugcacuugucugugaaucuuagcuggugcuagugucucuguccucucugggugcacacacguucuccuuuggacuuuuuaacuggaucuugcuuggaauuuuucccuuuccauauuugguuacugguuuggaaguuuauuucccuuuguuuuacuaaucauuuuguuccauuauuuuuggugguucuaguuagaaaauagcucccacugcauuuuggugcaacaauuuuaaaggccucuauaagauguuaucuucuguccugcuuguagacugagcuuuagguuguaccuuaauuacuaacauaaauaacuuuuuggagcaaggugcacaacacuauauauaauaugauuugauuuucuggaagguauacagcaguaagcauaauaaauugugaucuuuauuucuaaagaaauuauaagaguaugcuuauauauacuggaacuauuucuuuucuaauuuccugaaaccauuugcaggaaacuuaaggauggucuaucugagaagcaaaggagucaggaaggcuggaaaggagacuuauuucuuguuuuguaaacuuacugcucuguuugaauuuacccuaagcauauauuauuuuuaguuagacauauaagaaaauguguuuaacaauucauucauuuuuaucuuugguuuuguccauaguauguauuuaggaaguuucacaaugugaagaaagcgaagaguaaaaacagcaggugacugcauugacaaaaugaaagcaagcaaauuggacaaaccuagcauaaagaagacagaccagguuaugcauuuuuacuccuuacaaauauaaagacaagcccguccuaaauuaucccaguagaaaauuuugacaacuacaacaaaacagaaaacccaacaaaacaaauaaaaauuugaugcugaugacaugcgauaaagaaaagcagagcucuccaguaaaaaccaaaauuccugucuguuaaguuuacaaggauucuuccuuaggacuuucugagccaagacaauggacagcuaagagggcagcucuugaaauacuuucacaggauuugcuucucugcucauaaaauguaggaacaauucaaacuggagagcauuuccuacccauucacuggccugaagauucauagaguaggguuuuguguugcugucagcaggcauuuaucugagcacacauccauccauccucccucucucucucucucuccuucucucucucucucuuuccccccacacccgaugcaugcauacacucacacacuuuggaacuuagaaggccacucuucugaauaucaaaucaaguaaaaugaccauucuaagggugacaacucagggaaacucuggaaacacuggaaacaaauacugaaaauaaacuuacgugugggagagagaauaacauugaaagaagguauacauaguaaccaaaagagcuacuguuucauguuuauagguugggaacugaacagaaaguugaaaacacagcacacaugauuaaaaaauuuuuuccuuaaaaaccaaagagccauuuuucuuaaauuccugaucagauuuaauuaacuacauuucaaaugcagucaugcacugcauaaugacauuuuggucaacaaugaaccauaucaguggucccacagauuauaauggagcugaaaaauucuuaucaucuagugaugcuauaacgcccguacu

SEQ ID NO: 3 - RNA, 978 nt, Homo sapiens
uagucagaauccacuacucuaccacuaaugucucuuccauccggcucugcagcaccugagcaaaagaccucugcagcugaguccaaagagcauucccaugugaaccgagcaaccaaguaucaucggagugaguuuguuagauucuagccccauccugugcuaggccuuagguagaccucuuacagcucacaagaaaugcaguuuaugaggaaagaccaugaaucggggggcggcccggggaggguauuaccaaacagaucagcaucaggaacaucauucccagagagaaauuuggccaauugucaguucaaguacacaucucucccuccuuuuacagcauauugcaauagauuauagccaugcgaaauaauccauaaacuuagcuaauuccaccaaacagauaggaaagaagguagaguccuacaagagccuagucagaauaagaacuacaguaauuuugccaaaacccuguuaaguucuugaauaauucuggucaaaauggauuucaaucugaguuaacucacagucaacaauuuggcuguuuuucuugcuucucacucuacugccuuacucucuuccacaguguuaaguagccauuuaaauggguuuguucugcugcagguggcugagccugggauuuccaacuugggagacuacacaguggacucuauaaugauuaguggcagcauccaaugucucuuccaagucuaaaauuugugaguuucaaaguugacucuccccaaaccuggccuuugcugccucagauucugucacucuagcaaggcagagagagcaaaaggggcaagacaaaccucaucaacagcacagaaaucccagaaucacacacucucugguccagccaagccaaguguuuuuuuuuuuguuguuguuguuguuuuuuaaaucacccuccauuacucaacauucucguucccagaugaauuuuaaacuggaguugcaccaacugugagacagccu

SEQ ID NO: 4 - RNA, 781 nt, Homo sapiens
cuggguucaagaugcagaauggugccuacggcaaaaaaaaaaaaaaaaaacacccuccucccuucuuuaccauuugaauggacauuuuccuuaccugugaucccaacagaaacagauccagaccuaucaugugaaguccacguuccaggaucagaaguaaccaguuuauggacugagcuuacacgggaaagucuacccccgacuccuucuggauaguaacauacacagcugcauaaaaacgucuccaaggggacauacgaugcauuugcuuggugucccagccaagcuccccaccggcgaccucacuguuccuuagagcucaagagcucgucuccuaucaaucagagaaccccaucagcugugaccaacagagcuggagcccucuguggagggagcugaccccacacacaggacagagcagaauccugauuauuuuacaaacugcaaaccuucugaguaagaagacaaaaauauacauuccaagguaucuguaaagugcuuggaagaugcagacagcugcaccgaggggcucugauccauccacacgcugcgcuuugcugcggucacacacacggucucagucacgugaugguuuugcuuuuauuucuuaaacggcugagugauaauccagcuagugugcagucauuucauaccuuucaaugggcgucaccgcagugacgcugccccagccccaugcugagggccgacacaauucacggaacagauucaucauauuuggucuuuauguaaauaauaaauguuuuaaaauugccuaaauaua

SEQ ID NO: 5 - DNA, 2728 bp, Homo sapiens
aggaccgccgagctttgctgaggcatcatggtgggacttaaagaagtatcttggccgggcgcagtggctcacacctataatcccagaactttgggaggatgaggcaggaggatcaattgagtcacggagttcaagaccagcctgggcaacagagtgagactctgtctctacaacaaattttaaaaaaattagtcaggtatggtgacgtgcacgtatagtctcagctacttgggaggctgaggtgggaggatcacttgagctcgggaggtggaggttgcagtgagccatgattgcgccactcactctaacataggtgacagagtgagatcccgtctccaaaaacaaacacaaacaaactaaaagaagtatcagctgctacacatctggaatgacaacatatgcagaatacaaatgtaaatagaaaacatagaatataaattatgagttttagttgagtaacgctgacttggaattggaagaacatttgcaggcatcagtaatgggagagtagaaaatgtgagaaagaaaccttaagtcaattaagagaatacactctgcaaattaggggtggatccttgggttaatctgcagcctgcagttgtaccctgctagaagcagcttcgatgccactgaagttaatcttgggtcccagtaaatatcttctctcctctctattatccactgtgcaagatatatgtaaatactgccagatacattttttaaaaggcccgggtgctatcgtgtataggttgacattaatgtactcccagaatgcccaggcatggtatggggtggccaccctatggttcctgttttcttagacggaagaccactcctgcagaacatttattatcagcctaggccagtgtgaacatactgggtacattttaggattcagtttatctgttttgtttagggttggtgctaatttggaataagcaaaccattcatgatctgtatcacataatttggtttagaatctgtcaccttacctgttgcggtcactccctctgaatttggggaccccaagaccaagttttactcttctgctctttccacctccagtgctaaggcctagaggggcgcaccttaaatctgaatcaatccacaaagcccgacggacgccagtggcagggtttggtgggattttaatagtaacctacaaaaaaagtcaggaagatagggaatagggacgaattattctcttctactcttcaaattttcagtgttgctctcattgcatattctcaccttgaaatcactgctagagacttcccaagtccaaagggtaagaaactaccttcagactggcttgggaaatgtttagagctgccagggttgtatgtaaaatttccatggcaataaaccactgatacattttttgttctattccacctaggaaaaacaaagatccccaaagtccatttcgctccgaggtcagtggacacagctctgtgactgtcctgtgctgtgtgggtctgtagaagggccagtcatgggccatcgagctactcacagccaactgcacccaagtccaagcctggctctgttcccatacacagagacaggatgggggctgctgatctggcctgaagccttgctctgggcactgaaaacgggggctatttccttacctgaagatctggaagcagcatgttgacaaaagcaccaactgctctgccatcacgtcccactgggtgtcagtgggaaggcctaaccaaggcctgcctccagtggctatcaggcagacgggccagcagttcccctccaggagcaagggacccttcttacccttttgatcacatttccctctcttaaaggggcactgctgtgggaaggggtcatgccttggatcctacagtcatggactgtgggtgaaacaggggctcttgactcttcacttcctagccataactctgcccattggaccacccaccctccctgctgctggtctcctggctcacccatcaaatccaactgctttatctagaaaatacttttctccattctcatttccctttgctttcccactcacctctgtttttgtttctgttttattttgttccagacacccttttcagggaagtagatcagggaggcccaagagattaggcctgggtgggctgctatcgcttaagaacacgtctgcctctggggctcctccctaacagctggcctctggagctgggagatgcagctgcctggcagtctgcagaggcagattgtgttgttacgtgctggtcaccgccttgagccttaaaccacagtcagcaatgaacctggaggcagggcatctctggggatgatcgaccgcatctgctcaggttcttgcagggcagggcaggcagagatgtgtgtttggagccagaaagccttcctgccaacctgccatgcctcagtttccctatctgaaccaccttcataaaaacaacttacggctctcagagcagcacatttgtaaaaacctgaaaaatataaagaaaaacgtcactcacatttctcccatgaacattttcctattttatgtatcttttatgtaactgaatcacattgcatatacaattatgtgttccatttttaaacaataagcttcccttgttttaaaagtaataatccatgtttattatgtgttattgcatagaaatttcagacacaaaaaaagaaaggaaaaatgactccttattgctccattgagaaataataaatatgaatattattctgataaata

SEQ ID NO: 6 - DNA, 8559 bp, Homo sapiens
aattttttttttttttttttttttgagagaaagtctcactctgttgcccaggctagagtgcagtggtacagtcttggctcactgcaacctctgcctcccaggttcaagcgattcttgtgtctcagcctcccaagtagttgagattacaggcacgagccaccacacctggcgaatttttgtatttttagtagagagggggtttcaccatgttggccaggctggtctcaactcctgacctcaagtaatccacccatctcagcctcccaaagtgctgggattacaggcgtgagccacagcacctgccctggttgtcctactttcaatgatgctaagattaatcagtgtttcaggtgataacagactgatccttccattgtaaagctccaatcaacattttgtctaatgattttagccattaataatcataccctaagtcaattacatgctgcaaatgatgattagattctattattttttcattatctattttctttgacattcattagcttgaattctataaagaagaacttttccttctaagttaaggctatgtggttacacatacatgcctaaaagaaagcagaataaagataagtatttattttgattgccaaatatcagggtaaggagtaactgacctagttaattctaatggtgaccaaagtgtgatgacttttaaacattttattgattttcttttttgtatctttataattaatgcattttgaaataaattcaacacatttaaatcaattgcattcagtatatgttttctcttttgactctcatcttgcctccagtttggctaaagaaagactttttaggttaattcctttgtcctttgggcacaatctcattagtctttgatagctaccttgctttctaagtgatatggttaggctttgtgtccctacccaaatctcatcttgaattgtaatccccataatccccatcatccccacgtgtaaagggagagacgagatagaggtaacaatcatggtggcagtttctctcatgctgttctcatgatagtgagttctcacaagatctgatggttttataaagagctcttcccccttcacttggcattgtccttcttgccaccactttgtgaagaaggtgccttgcttcccctttgccttctaccatgattttaagttttctgaggcctccccagccacactgaactgtgagtcaattaaacctcttttcttcataaattacccagtttctggcagttccttatagcagtgtgaaaacagactaatacaccagggcaacaaaccgtcccaggctcatcttaaattgcctaaccttaaaactggagtcaggtgtccctccaaagtttcctagtcattgttagtgtggaatggtatttagggattatagtctatatgctaagtatgctcattttcaaggggttgtagaatagtttatattattatcctcaactcctaactcccttctcatttattattgtatgatttctagggcctcccagcaggcagaacacaattctccatcccagttccacgtttggccacgtgatgtgctttgaccaatgggcacatatcatgttaagtagaagcttttagagctgttaaggacagagctaagctttgtcctttgcttttccctaggccacaaggacagtctgttccaaacagggtcaattgcttcagcttgagtcctggaaaaagaagattgtagagaaaagactcagcagctgatctggagccaccaaaatggaatacaagccaaatatataatgcatatggtggcaaactactgaggtttttaaggttatctgttacttcttcaaagctgattgatacaggctgtgatgtcttctgggcctttttagtagacagataggaaaagcagctttgaaaagaggaaagcattgtgagttcaaactcaattcaaatagaacatttccaaatcagatagaacattataggacctgtacttaatttttaaaaactttatacatatatctcttttttctacactaaaaatcttaatttctatttacattagtataattactgatttgtatttcctataatataacatagtgtcaaaataacaaaatcattattttaaagtactaaagtttaaaacatatttgtagctatttttgtccttaagatatattctactgtttggtggaatattatgtttttaggttcagattgaaataattatttcctttatgtggttatatcactaatttgatatacagtaggttcatttccttatttctttttttttcttttagagacagcatctttctctgtcacccacgctagagtgcagtagcacaatcacagctcaccacagcctcgatctcccaggaccaagcaaacctcccacctcagcctcgtgagtagctgagactacaggcatgccaccatgcccagctaatttttatttatttttcttttttgtagaggcgtggccttcctatatggcctaggctggtcttgaactcctggtcttaagcaatcttcctgcctgggcctcccaaagtatggggattacaagtgtaaaccaccatgcccagctcagtaagttcatttatttccatttgttttccatttttagggaaggctattttagtgaattttatcttttgaaataaaacatttaaaatttcaaaatgaaatctatgtaataagctatacatagtaagagaagtctgttccattcctgttctacctattgttaatagtttcattagttaacagtttaacctgccagtgtttctgtcatacacaaaatgtagcatgttgcactagattgttctgcatcttacttttttcacttactatattttggagatgacagtacagagagatcaccatcattcctttatatcgctacagtgcctaccattgtgttatttatttagccaatcccctataaatgggcatttgttttcaatcatttttataatagttgtgaaataaataatacaatgcataaaaaagaaataacaccatgcataaagcatgtcctgtttttgcaactacagctttaacacaggttcccagtaacggggttgatgggtcaaagggcaaatatagaatttttctacatattgctgaatatgatgggtcaaaggctagatgtagaatttttctacatattgctgctccatagcagttgtatcatctcacagctccatcagcagtatgtagaatgcctatttccatacaacttcaataacagagtatgtggatgagtttatgtgattttgctaagggaagaagtgctatctttgggacaatctaatttgcattttaagttatactgagaaaagcttcatatttgaagaaccatttaaatttttcttctgggaactctgggttttttgtgtgccatttataaaattttgatatttgtattttaatttttaggggttccttttatatcagtgataatactctgtcagagatgtaacttacaaatatcctttcccaattagtcatttatctttggatttgtttagggtgttttattttttccatgcagacactcatttgatttatagtccagtttacagaagaacagatccatactttgttttttttttttttttttttttggcggggggaggtatggttttatttatttatttacctatttacatttagatctctgatccatttgaaattaattctcatggagaatatcaggttctgatccatttttccctcaaatggttcccagttgtaacaatattgattaagcattctccatggtttcaaatgctaccattttacacacacatacacacatacacgtgatttctaaatgaagttggcataatttccggactttatatactcttccattggcttgtctgtctattcatgtaccaatctcacattattttacttatagaggctttatagaacactataatatagggctataaccacttcatttctgccccgttagtgtattattaattctccattgtctcattcatttgatatttattctatgtattatatgttttatgattaatatgttgatacagaaatacatattacaatttattaaaacacacgtcaggacatatcctcttttaagaaatgaagtaggatatgtaatataaaaaagtttgaagatcactgattcagtgttttttgaacatgccagcatctttagatagctgtcctgggtggcagtagcacaatggagctgagattcttacatgtatctgattttggcatttgcctaatgctgaatgagattcttggcagagacaatgactcacctggatccaggggtaattttttaagtgctaatgagcaagtgtcaagatcccacaaaatcattaaaagtaacggctaaaactgcagttacttttgcaccaacctataaaaatactggacaagaacacctaggaaaatcatctttgatttggaaatgaagatcactttatcaggctctacaatggtttaaatgtgttcctcagaattcatgtataggaaattgagttcccagtataatggtgttgagaggtggtaggacctttaagaggtgtttgggtcatgaagactctgccaccctcacgaagatattagtcccattctcataggactgggttaattctcacagaagcaaatgagttcttgttctcatgggactagattagtaactgcaagagcaggttgttaaaaaatgaggccatcacttgtgttttgtctcttttgcacatacttgcttgctgctcctgcaggtgtttccacatgtgatgccattcactatgctttaatgtagcatgagggccttgccagaggtagctgcccaatgttgaacttcccaggctccagaactgggagccaagtaaacctcttttgtttataaattacccagtctcaggtgttctgttacagcaacagaaatagactaaaacagtctctattgtctcatctctcttaataaacttttgctcattatgggatatagattgctattatatcaattgagtaacaaagagattaggccatgaggggaaagtctggagattccctgctccagagagtagaacttttacaactaacatgctaatacggtttggttgtgtcgccacccaaatctcatcttgaattgtagttcccataatccccacatgttgtgggagagacacggtggcaggtaattgaatcatggaagtggttacctccatgctttcttttctcatgatagtgaatgagctcttatgagatctgatgattttataaagggctttccccgcttttgctcggcacttctgcttccggccatcaagtaaagaagaatgtgtttgcttccccttctgccatgattgtaagtttcctgaggcctccccagccatgcgaaactgagagtcaattaaacctctttcctttgtaaattacccagtcttgggcagtcctttacagcagcgtgagaacacactaatacgtgctttgttctagtctagattaagcaacttttgaggggtgtattgtttgactcatctgagtttttaatcaatgcttactaattcaagaggaacttatgtgcttttaggatataaggaggcatcaggaaatctggaaaatttcttaaaatcctataaggcagaccagtctttatatttccttatatcttagggaggccactgttaaaaagaggaggagggagttttaggagcagtaatattatgcattcatttgagactattaattttacatatgtcttgaggtttttattgctaaaaagttatataattttatgaagctacaaaacaaataaacattaaattccagcttatgtaattctacttaatcaagtattaaatgtgccaggcagtactctaggtaccaacgacctaaagatgtgttgtctctgcctccagcaagctcacaatacagagagatatacatggaaaaattgtaacagtacagctcagtaagtgccataagagaataaagaatataccaaaagcaccagagtataatatacagtagacatcagctttgaggaattgatgagttggaaagaattaagagaaggcgcaaggaattttggagttagaccttcagggagaaattgcatttggccatatgaggaacaatagcaacaacaacagagatgaatggaggttgggaagaagtactgtatctagataaaatggcatagatgttcactcgtttacacacacacacacacacacacacacaaacacacggcacaaaagaacctgacttgttctggatccaaaagcactatatggacagtacaataatctcatgtctccaatatgcttaggtacaattttaatgttttatgacatagatggctgcatgtttcagttattggacaaatgcatacttgagttattgtttattccattgtgtcagttctgcttctgatcaaaatccattcctatttgaaaatgcatctagtgaatttttttttttgagacagaatcttgctgtgttgcccaggctggagtgcagtggcacaatctcagctcattgcaacctccgcctcccacgttcaagtgattctcatgcctcagcctcctgagtagctgggactacaggtgcatgccaccatgcccagctactttttgtacttttagtagatacagggtttcaccacgttggctaggctggtttcaaactcctgacctcaggtgatccacccgtcttggcctcccaaagtgctgggattacaggcgtgagtcacagcgcccagccctctagtgcattttttaaaaaacataaacaccattctctcttttcaaatttagcacttgcccagaagtttgacatgttccctttttatttgtggtcattatttcctctttggtctcctttaaaaatagcacccctttgcacttgtctgtgaatcttagctggtgctagtgtctctgtcctctctgggtgcacacacgttctcctttggactttttaactggatcttgcttggaatttttccctttccatatttggttactggtttggaagtttatttccctttgttttactaatcattttgttccattatttttggtggttctagttagaaaatagctcccactgcattttggtgcaacaattttaaaggcctctataagatgttatcttctgtcctgcttgtagactgagctttaggttgtaccttaattactaacataaataactttttggagcaaggtgcacaacactatatataatatgatttgattttctggaaggtatacagcagtaagcataataaattgtgatctttatttctaaagaaattataagagtatgcttatatatactggaactatttcttttctaatttcctgaaaccatttgcaggaaacttaaggatggtctatctgagaagcaaaggagtcaggaaggctggaaaggagacttatttcttgttttgtaaacttactgctctgtttgaatttaccctaagcatatattatttttagttagacatataagaaaatgtgtttaacaattcattcatttttatctttggttttgtccatagtatgtatttaggaagtttcacaatgtgaagaaagcgaagagtaaaaacagcaggtgactgcattgacaaaatgaaagcaagcaaattggacaaacctagcataaagaagacagaccaggttatgcatttttactccttacaaatataaagacaagcccgtcctaaattatcccagtagaaaattttgacaactacaacaaaacagaaaacccaacaaaacaaataaaaatttgatgctgatgacatgcgataaagaaaagcagagctctccagtaaaaaccaaaattcctgtctgttaagtttacaaggattcttccttaggactttctgagccaagacaatggacagctaagagggcagctcttgaaatactttcacaggatttgcttctctgctcataaaatgtaggaacaattcaaactggagagcatttcctacccattcactggcctgaagattcatagagtagggttttgtgttgctgtcagcaggcatttatctgagcacacatccatccatcctccctctctctctctctctccttctctctctctctctttccccccacacccgatgcatgcatacactcacacactttggaacttagaaggccactcttctgaatatcaaatcaagtaaaatgaccattctaagggtgacaactcagggaaactctggaaacactggaaacaaatactgaaaataaacttacgtgtgggagagagaataacattgaaagaaggtatacatagtaaccaaaagagctactgtttcatgtttataggttgggaactgaacagaaagttgaaaacacagcacacatgattaaaaaattttttccttaaaaaccaaagagccatttttcttaaattcctgatcagatttaattaactacatttcaaatgcagtcatgcactgcataatgacattttggtcaacaatgaaccatatcagtggtcccacagattataatggagctgaaaaattcttatcatctagtgatgctataacgcccgtact

SEQ ID NO: 7 - DNA, 978 bp, Homo sapiens
tagtcagaatccactactctaccactaatgtctcttccatccggctctgcagcacctgagcaaaagacctctgcagctgagtccaaagagcattcccatgtgaaccgagcaaccaagtatcatcggagtgagtttgttagattctagccccatcctgtgctaggccttaggtagacctcttacagctcacaagaaatgcagtttatgaggaaagaccatgaatcggggggcggcccggggagggtattaccaaacagatcagcatcaggaacatcattcccagagagaaatttggccaattgtcagttcaagtacacatctctccctccttttacagcatattgcaatagattatagccatgcgaaataatccataaacttagctaattccaccaaacagataggaaagaaggtagagtcctacaagagcctagtcagaataagaactacagtaattttgccaaaaccctgttaagttcttgaataattctggtcaaaatggatttcaatctgagttaactcacagtcaacaatttggctgtttttcttgcttctcactctactgccttactctcttccacagtgttaagtagccatttaaatgggtttgttctgctgcaggtggctgagcctgggatttccaacttgggagactacacagtggactctataatgattagtggcagcatccaatgtctcttccaagtctaaaatttgtgagtttcaaagttgactctccccaaacctggcctttgctgcctcagattctgtcactctagcaaggcagagagagcaaaaggggcaagacaaacctcatcaacagcacagaaatcccagaatcacacactctctggtccagccaagccaagtgtttttttttttgttgttgttgttgttttttaaatcaccctccattactcaacattctcgttcccagatgaattttaaactggagttgcaccaactgtgagacagcct

SEQ ID NO: 8 - DNA, 781 bp, Homo sapiens
ctgggttcaagatgcagaatggtgcctacggcaaaaaaaaaaaaaaaaaacaccctcctcccttctttaccatttgaatggacattttccttacctgtgatcccaacagaaacagatccagacctatcatgtgaagtccacgttccaggatcagaagtaaccagtttatggactgagcttacacgggaaagtctacccccgactccttctggatagtaacatacacagctgcataaaaacgtctccaaggggacatacgatgcatttgcttggtgtcccagccaagctccccaccggcgacctcactgttccttagagctcaagagctcgtctcctatcaatcagagaaccccatcagctgtgaccaacagagctggagccctctgtggagggagctgaccccacacacaggacagagcagaatcctgattattttacaaactgcaaaccttctgagtaagaagacaaaaatatacattccaaggtatctgtaaagtgcttggaagatgcagacagctgcaccgaggggctctgatccatccacacgctgcgctttgctgcggtcacacacacggtctcagtcacgtgatggttttgcttttatttcttaaacggctgagtgataatccagctagtgtgcagtcatttcatacctttcaatgggcgtcaccgcagtgacgctgccccagccccatgctgagggccgacacaattcacggaacagattcatcatatttggtctttatgtaaataataaatgttttaaaattgcctaaatata